European Patent Specification EP 3 368 557 B1, published March 25, 2026. Title: NEW POLYPEPTIDE. Applicant: AFFIBODY AB. The sequence listing filed with the application follows.

SEQUENCE LISTING (74 sequences)

SEQ ID NO: 1 - protein, 58 aa, Artificial Sequence
  Engineered PD-L1 binding polypeptide
VDAKYAKERTVAVWEIVQLPNLTAWQKGAFINKLHDDPSQSSELLSEAKKLNDSQAPK

SEQ ID NO: 2 - protein, 58 aa, Artificial Sequence
  Engineered PD-L1 binding polypeptide
VDAKYAKERTWAVWEIMDLPNLTAGQRGAFINKLHDDPSQSSELLSEAKKLNDSQAPK

SEQ ID NO: 3 - protein, 58 aa, Artificial Sequence
  Engineered PD-L1 binding polypeptide
VDAKYAKERTIAVWEIMDLPNLTSWQRGAFIDKLHDDPSQSSELLSEAKKLNDSQAPK

SEQ ID NO: 4 - protein, 58 aa, Artificial Sequence
  Engineered PD-L1 binding polypeptide
VDAKYAKERTMATWEIVQLPNLTARQKGAFIWKLHDDPSQSSELLSEAKKLNDSQAPK

SEQ ID NO: 5 - protein, 61 aa, Artificial Sequence
  Engineered PD-L1 binding polypeptide
AEAKYAKERTVAVWEIVQLPNLTAWQKGAFINKLHDDPSQSSELLSEAKKLNDSQAPKVDC

SEQ ID NO: 6 - protein, 16 aa, Artificial Sequence
  Linker
GGGGSLVPRGSGGGGS

SEQ ID NO: 7 - protein, 6 aa, Artificial Sequence
  Linker
GSGSGS

SEQ ID NO: 8 - protein, 8 aa, Artificial Sequence
  Linker
GSGSGSGS

SEQ ID NO: 9 - protein, 16 aa, Artificial Sequence
  Linker
GSGSGSGSGSGSGSGS

SEQ ID NO: 10 - protein, 11 aa, Artificial Sequence
  Linker
GGSGGHMGSGG

SEQ ID NO: 11 - protein, 11 aa, Artificial Sequence
  Linker
GGSGGSGGSGG

SEQ ID NO: 12 - protein, 5 aa, Artificial Sequence
  Linker
GGSGG

SEQ ID NO: 13 - protein, 8 aa, Artificial Sequence
  Linker
GGSGGGGG

SEQ ID NO: 14 - protein, 18 aa, Artificial Sequence
  Linker
GGGSEGGGSEGGGSEGGG

SEQ ID NO: 15 - protein, 8 aa, Artificial Sequence
  Linker
AAGAATAA

SEQ ID NO: 16 - protein, 5 aa, Artificial Sequence
  Linker
GGGGG

SEQ ID NO: 17 - protein, 5 aa, Artificial Sequence
  Linker
GGSSG

SEQ ID NO: 18 - protein, 11 aa, Artificial Sequence
  Linker
GSGGGTGGGSG

SEQ ID NO: 19 - protein, 11 aa, Artificial Sequence
  Linker
GSGGGTGGGSG

SEQ ID NO: 20 - protein, 12 aa, Artificial Sequence
  Linker
GSGSGSGSGGSG

SEQ ID NO: 21 - protein, 14 aa, Artificial Sequence
  Linker
GSGGSGGSGGSGGS

SEQ ID NO: 22 - protein, 14 aa, Artificial Sequence
  Linker
GSGGSGSGGSGGSG

SEQ ID NO: 23 - protein, 29 aa, ARTIFICIAL SEQUENCE
  Engineered PDL1 binding polypeptide
  misc_feature (4)..(4): Xaa can be any naturally occurring amino acid
  misc_feature (6)..(6): Xaa can be any naturally occurring amino acid
  misc_feature (10)..(11): Xaa can be any naturally occurring amino acid
  misc_feature (16)..(18): Xaa can be any naturally occurring amino acid
  misc_feature (20)..(20): Xaa can be any naturally occurring amino acid
  misc_feature (25)..(26): Xaa can be any naturally occurring amino acid
ERTXAXWEIXXLPNLXXXQXGAFIXXLHD

SEQ ID NO: 24 - protein, 49 aa, ARTIFICIAL SEQUENCE
  Engineered PDL1 binding polypeptide
  misc_feature (5)..(5): Xaa can be any naturally occurring amino acid
  misc_feature (7)..(7): Xaa can be any naturally occurring amino acid
  misc_feature (11)..(12): Xaa can be any naturally occurring amino acid
  misc_feature (17)..(19): Xaa can be any naturally occurring amino acid
  misc_feature (21)..(21): Xaa can be any naturally occurring amino acid
  misc_feature (26)..(27): Xaa can be any naturally occurring amino acid
  misc_feature (36)..(37): Xaa can be any naturally occurring amino acid
  misc_feature (40)..(40): Xaa can be any naturally occurring amino acid
  misc_feature (46)..(48): Xaa can be any naturally occurring amino acid
KERTXAXWEIXXLPNLXXXQXGAFIXXLHDDPSQSXXLLXEAKKLXXXQ

SEQ ID NO: 25 - protein, 53 aa, ARTIFICIAL SEQUENCE
  Engineered PDL1 binding polypeptide
  misc_feature (7)..(7): Xaa can be any naturally occurring amino acid
  misc_feature (9)..(9): Xaa can be any naturally occurring amino acid
  misc_feature (13)..(14): Xaa can be any naturally occurring amino acid
  misc_feature (19)..(21): Xaa can be any naturally occurring amino acid
  misc_feature (23)..(23): Xaa can be any naturally occurring amino acid
  misc_feature (28)..(29): Xaa can be any naturally occurring amino acid
  misc_feature (38)..(39): Xaa can be any naturally occurring amino acid
  misc_feature (42)..(42): Xaa can be any naturally occurring amino acid
  misc_feature (48)..(50): Xaa can be any naturally occurring amino acid
YAKERTXAXWEIXXLPNLXXXQXGAFIXXLHDDPSQSXXLLXEAKKLXXXQAP

SEQ ID NO: 26 - protein, 53 aa, ARTIFICIAL SEQUENCE
  Engineered PDL1 binding polypeptide
  misc_feature (7)..(7): Xaa can be any naturally occurring amino acid
  misc_feature (9)..(9): Xaa can be any naturally occurring amino acid
  misc_feature (13)..(14): Xaa can be any naturally occurring amino acid
  misc_feature (19)..(21): Xaa can be any naturally occurring amino acid
  misc_feature (23)..(23): Xaa can be any naturally occurring amino acid
  misc_feature (28)..(29): Xaa can be any naturally occurring amino acid
  misc_feature (38)..(39): Xaa can be any naturally occurring amino acid
  misc_feature (42)..(42): Xaa can be any naturally occurring amino acid
  misc_feature (48)..(50): Xaa can be any naturally occurring amino acid
FNKERTXAXWEIXXLPNLXXXQXGAFIXXLHDDPSQSXXLLXEAKKLXXXQAP

SEQ ID NO: 27 - protein, 53 aa, ARTIFICIAL SEQUENCE
  Engineered PDL1 binding polypeptide
  misc_feature (7)..(7): Xaa can be any naturally occurring amino acid
  misc_feature (9)..(9): Xaa can be any naturally occurring amino acid
  misc_feature (13)..(14): Xaa can be any naturally occurring amino acid
  misc_feature (19)..(21): Xaa can be any naturally occurring amino acid
  misc_feature (23)..(23): Xaa can be any naturally occurring amino acid
  misc_feature (28)..(29): Xaa can be any naturally occurring amino acid
  misc_feature (42)..(42): Xaa can be any naturally occurring amino acid
FNKERTXAXWEIXXLPNLXXXQXGAFIXXLHDDPSQSANLLXEAKKLNDAQAP

SEQ ID NO: 28 - protein, 53 aa, ARTIFICIAL SEQUENCE
  Engineered PDL1 binding polypeptide
  misc_feature (7)..(7): Xaa can be any naturally occurring amino acid
  misc_feature (9)..(9): Xaa can be any naturally occurring amino acid
  misc_feature (13)..(14): Xaa can be any naturally occurring amino acid
  misc_feature (19)..(21): Xaa can be any naturally occurring amino acid
  misc_feature (23)..(23): Xaa can be any naturally occurring amino acid
  misc_feature (28)..(29): Xaa can be any naturally occurring amino acid
  misc_feature (42)..(42): Xaa can be any naturally occurring amino acid
FAKERTXAXWEIXXLPNLXXXQXGAFIXXLHDDPSQSSELLXEAKKLSESQAP

SEQ ID NO: 29 - protein, 53 aa, ARTIFICIAL SEQUENCE
  Engineered PDL1 binding polypeptide
  misc_feature (7)..(7): Xaa can be any naturally occurring amino acid
  misc_feature (9)..(9): Xaa can be any naturally occurring amino acid
  misc_feature (13)..(14): Xaa can be any naturally occurring amino acid
  misc_feature (19)..(21): Xaa can be any naturally occurring amino acid
  misc_feature (23)..(23): Xaa can be any naturally occurring amino acid
  misc_feature (28)..(29): Xaa can be any naturally occurring amino acid
  misc_feature (42)..(42): Xaa can be any naturally occurring amino acid
FAKERTXAXWEIXXLPNLXXXQXGAFIXXLHDDPSQSSELLXEAKKLNDSQAP

SEQ ID NO: 30 - protein, 53 aa, ARTIFICIAL SEQUENCE
  Engineered PDL1 binding polypeptide
  misc_feature (7)..(7): Xaa can be any naturally occurring amino acid
  misc_feature (9)..(9): Xaa can be any naturally occurring amino acid
  misc_feature (13)..(14): Xaa can be any naturally occurring amino acid
  misc_feature (19)..(21): Xaa can be any naturally occurring amino acid
  misc_feature (23)..(23): Xaa can be any naturally occurring amino acid
  misc_feature (28)..(29): Xaa can be any naturally occurring amino acid
  misc_feature (42)..(42): Xaa can be any naturally occurring amino acid
YAKERTXAXWEIXXLPNLXXXQXGAFIXXLHDDPSQSSELLXEAKKLNDSQAP

SEQ ID NO: 31 - protein, 58 aa, ARTIFICIAL SEQUENCE
  Engineered PDL1 binding polypeptide
  misc_feature (11)..(11): Xaa can be any naturally occurring amino acid
  misc_feature (13)..(13): Xaa can be any naturally occurring amino acid
  misc_feature (17)..(18): Xaa can be any naturally occurring amino acid
  misc_feature (23)..(25): Xaa can be any naturally occurring amino acid
  misc_feature (27)..(27): Xaa can be any naturally occurring amino acid
  misc_feature (32)..(33): Xaa can be any naturally occurring amino acid
ADNNFNKERTXAXWEIXXLPNLXXXQXGAFIXXLHDDPSQSANLLSEAKKLNESQAPK

SEQ ID NO: 32 - protein, 58 aa, ARTIFICIAL SEQUENCE
  Engineered PDL1 binding polypeptide
  misc_feature (11)..(11): Xaa can be any naturally occurring amino acid
  misc_feature (13)..(13): Xaa can be any naturally occurring amino acid
  misc_feature (17)..(18): Xaa can be any naturally occurring amino acid
  misc_feature (23)..(25): Xaa can be any naturally occurring amino acid
  misc_feature (27)..(27): Xaa can be any naturally occurring amino acid
  misc_feature (32)..(33): Xaa can be any naturally occurring amino acid
ADNKFNKERTXAXWEIXXLPNLXXXQXGAFIXXLHDDPSQSANLLAEAKKLNDAQAPK

SEQ ID NO: 33 - protein, 58 aa, ARTIFICIAL SEQUENCE
  Engineered PDL1 binding polypeptide
  misc_feature (11)..(11): Xaa can be any naturally occurring amino acid
  misc_feature (13)..(13): Xaa can be any naturally occurring amino acid
  misc_feature (17)..(18): Xaa can be any naturally occurring amino acid
  misc_feature (23)..(25): Xaa can be any naturally occurring amino acid
  misc_feature (27)..(27): Xaa can be any naturally occurring amino acid
  misc_feature (32)..(33): Xaa can be any naturally occurring amino acid
ADNKFNKERTXAXWEIXXLPNLXXXQXGAFIXXLHDDPSVSKEILAEAKKLNDAQAPK

SEQ ID NO: 34 - protein, 61 aa, ARTIFICIAL SEQUENCE
  Engineered PDL1 binding polypeptide
  misc_feature (14)..(14): Xaa can be any naturally occurring amino acid
  misc_feature (16)..(16): Xaa can be any naturally occurring amino acid
  misc_feature (20)..(21): Xaa can be any naturally occurring amino acid
  misc_feature (26)..(28): Xaa can be any naturally occurring amino acid
  misc_feature (30)..(30): Xaa can be any naturally occurring amino acid
  misc_feature (35)..(36): Xaa can be any naturally occurring amino acid
ADAQQNNFNKERTXAXWEIXXLPNLXXXQXGAFIXXLHDDPSQSTNVLGEAKKLNESQAPK

SEQ ID NO: 35 - protein, 56 aa, ARTIFICIAL SEQUENCE
  Engineered PDL1 binding polypeptide
  misc_feature (9)..(9): Xaa can be any naturally occurring amino acid
  misc_feature (11)..(11): Xaa can be any naturally occurring amino acid
  misc_feature (15)..(16): Xaa can be any naturally occurring amino acid
  misc_feature (21)..(23): Xaa can be any naturally occurring amino acid
  misc_feature (25)..(25): Xaa can be any naturally occurring amino acid
  misc_feature (30)..(31): Xaa can be any naturally occurring amino acid
AQHDEERTXAXWEIXXLPNLXXXQXGAFIXXLHDDPSQSANVLGEAQKLNDSQAPK

SEQ ID NO: 36 - protein, 58 aa, ARTIFICIAL SEQUENCE
  Engineered PDL1 binding polypeptide
  misc_feature (11)..(11): Xaa can be any naturally occurring amino acid
  misc_feature (13)..(13): Xaa can be any naturally occurring amino acid
  misc_feature (17)..(18): Xaa can be any naturally occurring amino acid
  misc_feature (23)..(25): Xaa can be any naturally occurring amino acid
  misc_feature (27)..(27): Xaa can be any naturally occurring amino acid
  misc_feature (32)..(33): Xaa can be any naturally occurring amino acid
VDNKFNKERTXAXWEIXXLPNLXXXQXGAFIXXLHDDPSQSANLLAEAKKLNDAQAPK

SEQ ID NO: 37 - protein, 58 aa, ARTIFICIAL SEQUENCE
  Engineered PDL1 binding polypeptide
  misc_feature (11)..(11): Xaa can be any naturally occurring amino acid
  misc_feature (13)..(13): Xaa can be any naturally occurring amino acid
  misc_feature (17)..(18): Xaa can be any naturally occurring amino acid
  misc_feature (23)..(25): Xaa can be any naturally occurring amino acid
  misc_feature (27)..(27): Xaa can be any naturally occurring amino acid
  misc_feature (32)..(33): Xaa can be any naturally occurring amino acid
AEAKYAKERTXAXWEIXXLPNLXXXQXGAFIXXLHDDPSESSELLSEAKKLNKSQAPK

SEQ ID NO: 38 - protein, 58 aa, ARTIFICIAL SEQUENCE
  Engineered PDL1 binding polypeptide
  misc_feature (11)..(11): Xaa can be any naturally occurring amino acid
  misc_feature (13)..(13): Xaa can be any naturally occurring amino acid
  misc_feature (17)..(18): Xaa can be any naturally occurring amino acid
  misc_feature (23)..(25): Xaa can be any naturally occurring amino acid
  misc_feature (27)..(27): Xaa can be any naturally occurring amino acid
  misc_feature (32)..(33): Xaa can be any naturally occurring amino acid
VDAKYAKERTXAXWEIXXLPNLXXXQXGAFIXXLHDDPSQSSELLAEAKKLNDAQAPK

SEQ ID NO: 39 - protein, 58 aa, ARTIFICIAL SEQUENCE
  Engineered PDL1 binding polypeptide
  misc_feature (11)..(11): Xaa can be any naturally occurring amino acid
  misc_feature (13)..(13): Xaa can be any naturally occurring amino acid
  misc_feature (17)..(18): Xaa can be any naturally occurring amino acid
  misc_feature (23)..(25): Xaa can be any naturally occurring amino acid
  misc_feature (27)..(27): Xaa can be any naturally occurring amino acid
  misc_feature (32)..(33): Xaa can be any naturally occurring amino acid
VDAKYAKERTXAXWEIXXLPNLXXXQXGAFIXXLHDDPSQSSELLAEAKKLNDSQAPK

SEQ ID NO: 40 - protein, 58 aa, ARTIFICIAL SEQUENCE
  Engineered PDL1 binding polypeptide
  misc_feature (11)..(11): Xaa can be any naturally occurring amino acid
  misc_feature (13)..(13): Xaa can be any naturally occurring amino acid
  misc_feature (17)..(18): Xaa can be any naturally occurring amino acid
  misc_feature (23)..(25): Xaa can be any naturally occurring amino acid
  misc_feature (27)..(27): Xaa can be any naturally occurring amino acid
  misc_feature (32)..(33): Xaa can be any naturally occurring amino acid
AEAKYAKERTXAXWEIXXLPNLXXXQXGAFIXXLHDDPSQSSELLSEAKKLNDSQAPK

SEQ ID NO: 41 - protein, 57 aa, ARTIFICIAL SEQUENCE
  Engineered PDL1 binding polypeptide
  misc_feature (11)..(11): Xaa can be any naturally occurring amino acid
  misc_feature (13)..(13): Xaa can be any naturally occurring amino acid
  misc_feature (17)..(18): Xaa can be any naturally occurring amino acid
  misc_feature (23)..(25): Xaa can be any naturally occurring amino acid
  misc_feature (27)..(27): Xaa can be any naturally occurring amino acid
  misc_feature (32)..(33): Xaa can be any naturally occurring amino acid
AEAKYAKERTXAXWEIXXLPNLXXXQXGAFIXXLHDDPSQSSELLSEAKKLNDSQAP

SEQ ID NO: 42 - protein, 58 aa, ARTIFICIAL SEQUENCE
  Engineered PDL1 binding polypeptide
  misc_feature (11)..(11): Xaa can be any naturally occurring amino acid
  misc_feature (13)..(13): Xaa can be any naturally occurring amino acid
  misc_feature (17)..(18): Xaa can be any naturally occurring amino acid
  misc_feature (23)..(25): Xaa can be any naturally occurring amino acid
  misc_feature (27)..(27): Xaa can be any naturally occurring amino acid
  misc_feature (32)..(33): Xaa can be any naturally occurring amino acid
AEAKFAKERTXAXWEIXXLPNLXXXQXGAFIXXLHDDPSQSSELLSEAKKLNDSQAPK

SEQ ID NO: 43 - protein, 57 aa, ARTIFICIAL SEQUENCE
  Engineered PDL1 binding polypeptide
  misc_feature (11)..(11): Xaa can be any naturally occurring amino acid
  misc_feature (13)..(13): Xaa can be any naturally occurring amino acid
  misc_feature (17)..(18): Xaa can be any naturally occurring amino acid
  misc_feature (23)..(25): Xaa can be any naturally occurring amino acid
  misc_feature (27)..(27): Xaa can be any naturally occurring amino acid
  misc_feature (32)..(33): Xaa can be any naturally occurring amino acid
AEAKFAKERTXAXWEIXXLPNLXXXQXGAFIXXLHDDPSQSSELLSEAKKLNDSQAP

SEQ ID NO: 44 - protein, 58 aa, ARTIFICIAL SEQUENCE
  Engineered PDL1 binding polypeptide
  misc_feature (11)..(11): Xaa can be any naturally occurring amino acid
  misc_feature (13)..(13): Xaa can be any naturally occurring amino acid
  misc_feature (17)..(18): Xaa can be any naturally occurring amino acid
  misc_feature (23)..(25): Xaa can be any naturally occurring amino acid
  misc_feature (27)..(27): Xaa can be any naturally occurring amino acid
  misc_feature (32)..(33): Xaa can be any naturally occurring amino acid
AEAKYAKERTXAXWEIXXLPNLXXXQXGAFIXXLHDDPSQSSELLAEAKKLNDAQAPK

SEQ ID NO: 45 - protein, 58 aa, ARTIFICIAL SEQUENCE
  Engineered PDL1 binding polypeptide
  misc_feature (11)..(11): Xaa can be any naturally occurring amino acid
  misc_feature (13)..(13): Xaa can be any naturally occurring amino acid
  misc_feature (17)..(18): Xaa can be any naturally occurring amino acid
  misc_feature (23)..(25): Xaa can be any naturally occurring amino acid
  misc_feature (27)..(27): Xaa can be any naturally occurring amino acid
  misc_feature (32)..(33): Xaa can be any naturally occurring amino acid
AEAKYAKERTXAXWEIXXLPNLXXXQXGAFIXXLHDDPSQSSELLSEAKKLSESQAPK

SEQ ID NO: 46 - protein, 57 aa, ARTIFICIAL SEQUENCE
  Engineered PDL1 binding polypeptide
  misc_feature (11)..(11): Xaa can be any naturally occurring amino acid
  misc_feature (13)..(13): Xaa can be any naturally occurring amino acid
  misc_feature (17)..(18): Xaa can be any naturally occurring amino acid
  misc_feature (23)..(25): Xaa can be any naturally occurring amino acid
  misc_feature (27)..(27): Xaa can be any naturally occurring amino acid
  misc_feature (32)..(33): Xaa can be any naturally occurring amino acid
AEAKYAKERTXAXWEIXXLPNLXXXQXGAFIXXLHDDPSQSSELLSEAKKLSESQAP

SEQ ID NO: 47 - protein, 58 aa, ARTIFICIAL SEQUENCE
  Engineered PDL1 binding polypeptide
  misc_feature (11)..(11): Xaa can be any naturally occurring amino acid
  misc_feature (13)..(13): Xaa can be any naturally occurring amino acid
  misc_feature (17)..(18): Xaa can be any naturally occurring amino acid
  misc_feature (23)..(25): Xaa can be any naturally occurring amino acid
  misc_feature (27)..(27): Xaa can be any naturally occurring amino acid
  misc_feature (32)..(33): Xaa can be any naturally occurring amino acid
AEAKFAKERTXAXWEIXXLPNLXXXQXGAFIXXLHDDPSQSSELLSEAKKLSESQAPK

SEQ ID NO: 48 - protein, 57 aa, ARTIFICIAL SEQUENCE
  Engineered PDL1 binding polypeptide
  misc_feature (11)..(11): Xaa can be any naturally occurring amino acid
  misc_feature (13)..(13): Xaa can be any naturally occurring amino acid
  misc_feature (17)..(18): Xaa can be any naturally occurring amino acid
  misc_feature (23)..(25): Xaa can be any naturally occurring amino acid
  misc_feature (27)..(27): Xaa can be any naturally occurring amino acid
  misc_feature (32)..(33): Xaa can be any naturally occurring amino acid
AEAKFAKERTXAXWEIXXLPNLXXXQXGAFIXXLHDDPSQSSELLSEAKKLSESQAP

SEQ ID NO: 49 - protein, 58 aa, ARTIFICIAL SEQUENCE
  Engineered PDL1 binding polypeptide
  misc_feature (11)..(11): Xaa can be any naturally occurring amino acid
  misc_feature (13)..(13): Xaa can be any naturally occurring amino acid
  misc_feature (17)..(18): Xaa can be any naturally occurring amino acid
  misc_feature (23)..(25): Xaa can be any naturally occurring amino acid
  misc_feature (27)..(27): Xaa can be any naturally occurring amino acid
  misc_feature (32)..(33): Xaa can be any naturally occurring amino acid
AEAKYAKERTXAXWEIXXLPNLXXXQXGAFIXXLHDDPSQSSELLAEAKKLSEAQAPK

SEQ ID NO: 50 - protein, 58 aa, ARTIFICIAL SEQUENCE
  Engineered PDL1 binding polypeptide
  misc_feature (11)..(11): Xaa can be any naturally occurring amino acid
  misc_feature (13)..(13): Xaa can be any naturally occurring amino acid
  misc_feature (17)..(18): Xaa can be any naturally occurring amino acid
  misc_feature (23)..(25): Xaa can be any naturally occurring amino acid
  misc_feature (27)..(27): Xaa can be any naturally occurring amino acid
  misc_feature (32)..(33): Xaa can be any naturally occurring amino acid
AEAKYAKERTXAXWEIXXLPNLXXXQXGAFIXXLHDQPEQSSELLSEAKKLSESQAPK

SEQ ID NO: 51 - protein, 58 aa, ARTIFICIAL SEQUENCE
  Engineered PDL1 binding polypeptide
  misc_feature (11)..(11): Xaa can be any naturally occurring amino acid
  misc_feature (13)..(13): Xaa can be any naturally occurring amino acid
  misc_feature (17)..(18): Xaa can be any naturally occurring amino acid
  misc_feature (23)..(25): Xaa can be any naturally occurring amino acid
  misc_feature (27)..(27): Xaa can be any naturally occurring amino acid
  misc_feature (32)..(33): Xaa can be any naturally occurring amino acid
AEAKYAKERTXAXWEIXXLPNLXXXQXGAFIXXLHDDPSQSSELLSEAKKLESSQAPK

SEQ ID NO: 52 - protein, 57 aa, ARTIFICIAL SEQUENCE
  Engineered PDL1 binding polypeptide
  misc_feature (11)..(11): Xaa can be any naturally occurring amino acid
  misc_feature (13)..(13): Xaa can be any naturally occurring amino acid
  misc_feature (17)..(18): Xaa can be any naturally occurring amino acid
  misc_feature (23)..(25): Xaa can be any naturally occurring amino acid
  misc_feature (27)..(27): Xaa can be any naturally occurring amino acid
  misc_feature (32)..(33): Xaa can be any naturally occurring amino acid
AEAKYAKERTXAXWEIXXLPNLXXXQXGAFIXXLHDDPSQSSELLSEAKKLESSQAP

SEQ ID NO: 53 - protein, 58 aa, ARTIFICIAL SEQUENCE
  Engineered PDL1 binding polypeptide
  misc_feature (11)..(11): Xaa can be any naturally occurring amino acid
  misc_feature (13)..(13): Xaa can be any naturally occurring amino acid
  misc_feature (17)..(18): Xaa can be any naturally occurring amino acid
  misc_feature (23)..(25): Xaa can be any naturally occurring amino acid
  misc_feature (27)..(27): Xaa can be any naturally occurring amino acid
  misc_feature (32)..(33): Xaa can be any naturally occurring amino acid
AEAKYAKERTXAXWEIXXLPNLXXXQXGAFIXXLHDDPSQSSELLAEAKKLESAQAPK

SEQ ID NO: 54 - protein, 58 aa, ARTIFICIAL SEQUENCE
  Engineered PDL1 binding polypeptide
  misc_feature (11)..(11): Xaa can be any naturally occurring amino acid
  misc_feature (13)..(13): Xaa can be any naturally occurring amino acid
  misc_feature (17)..(18): Xaa can be any naturally occurring amino acid
  misc_feature (23)..(25): Xaa can be any naturally occurring amino acid
  misc_feature (27)..(27): Xaa can be any naturally occurring amino acid
  misc_feature (32)..(33): Xaa can be any naturally occurring amino acid
AEAKYAKERTXAXWEIXXLPNLXXXQXGAFIXXLHDQPEQSSELLSEAKKLESSQAPK

SEQ ID NO: 55 - protein, 58 aa, ARTIFICIAL SEQUENCE
  Engineered PDL1 binding polypeptide
  misc_feature (11)..(11): Xaa can be any naturally occurring amino acid
  misc_feature (13)..(13): Xaa can be any naturally occurring amino acid
  misc_feature (17)..(18): Xaa can be any naturally occurring amino acid
  misc_feature (23)..(25): Xaa can be any naturally occurring amino acid
  misc_feature (27)..(27): Xaa can be any naturally occurring amino acid
  misc_feature (32)..(33): Xaa can be any naturally occurring amino acid
AEAKYAKERTXAXWEIXXLPNLXXXQXGAFIXXLHDDPSQSSELLSEAKKLSDSQAPK

SEQ ID NO: 56 - protein, 57 aa, ARTIFICIAL SEQUENCE
  Engineered PDL1 binding polypeptide
  misc_feature (11)..(11): Xaa can be any naturally occurring amino acid
  misc_feature (13)..(13): Xaa can be any naturally occurring amino acid
  misc_feature (17)..(18): Xaa can be any naturally occurring amino acid
  misc_feature (23)..(25): Xaa can be any naturally occurring amino acid
  misc_feature (27)..(27): Xaa can be any naturally occurring amino acid
  misc_feature (32)..(33): Xaa can be any naturally occurring amino acid
AEAKYAKERTXAXWEIXXLPNLXXXQXGAFIXXLHDDPSQSSELLSEAKKLSDSQAP

SEQ ID NO: 57 - protein, 58 aa, ARTIFICIAL SEQUENCE
  Engineered PDL1 binding polypeptide
  misc_feature (11)..(11): Xaa can be any naturally occurring amino acid
  misc_feature (13)..(13): Xaa can be any naturally occurring amino acid
  misc_feature (17)..(18): Xaa can be any naturally occurring amino acid
  misc_feature (23)..(25): Xaa can be any naturally occurring amino acid
  misc_feature (27)..(27): Xaa can be any naturally occurring amino acid
  misc_feature (32)..(33): Xaa can be any naturally occurring amino acid
AEAKYAKERTXAXWEIXXLPNLXXXQXGAFIXXLHDDPSQSSELLAEAKKLSDSQAPK

SEQ ID NO: 58 - protein, 58 aa, ARTIFICIAL SEQUENCE
  Engineered PDL1 binding polypeptide
  misc_feature (11)..(11): Xaa can be any naturally occurring amino acid
  misc_feature (13)..(13): Xaa can be any naturally occurring amino acid
  misc_feature (17)..(18): Xaa can be any naturally occurring amino acid
  misc_feature (23)..(25): Xaa can be any naturally occurring amino acid
  misc_feature (27)..(27): Xaa can be any naturally occurring amino acid
  misc_feature (32)..(33): Xaa can be any naturally occurring amino acid
AEAKYAKERTXAXWEIXXLPNLXXXQXGAFIXXLHDDPSQSSELLAEAKKLSDAQAPK

SEQ ID NO: 59 - protein, 58 aa, ARTIFICIAL SEQUENCE
  Engineered PDL1 binding polypeptide
  misc_feature (11)..(11): Xaa can be any naturally occurring amino acid
  misc_feature (13)..(13): Xaa can be any naturally occurring amino acid
  misc_feature (17)..(18): Xaa can be any naturally occurring amino acid
  misc_feature (23)..(25): Xaa can be any naturally occurring amino acid
  misc_feature (27)..(27): Xaa can be any naturally occurring amino acid
  misc_feature (32)..(33): Xaa can be any naturally occurring amino acid
AEAKYAKERTXAXWEIXXLPNLXXXQXGAFIXXLHDQPEQSSELLSEAKKLSDSQAPK

SEQ ID NO: 60 - protein, 58 aa, ARTIFICIAL SEQUENCE
  Engineered PDL1 binding polypeptide
  misc_feature (11)..(11): Xaa can be any naturally occurring amino acid
  misc_feature (13)..(13): Xaa can be any naturally occurring amino acid
  misc_feature (17)..(18): Xaa can be any naturally occurring amino acid
  misc_feature (23)..(25): Xaa can be any naturally occurring amino acid
  misc_feature (27)..(27): Xaa can be any naturally occurring amino acid
  misc_feature (32)..(33): Xaa can be any naturally occurring amino acid
VDAKYAKERTXAXWEIXXLPNLXXXQXGAFIXXLHDDPSQSSELLSEAKKLNDSQAPK

SEQ ID NO: 61 - protein, 58 aa, ARTIFICIAL SEQUENCE; identical to SEQ ID NO: 38
  Engineered PDL1 binding polypeptide
  misc_feature (11)..(11): Xaa can be any naturally occurring amino acid
  misc_feature (13)..(13): Xaa can be any naturally occurring amino acid
  misc_feature (17)..(18): Xaa can be any naturally occurring amino acid
  misc_feature (23)..(25): Xaa can be any naturally occurring amino acid
  misc_feature (27)..(27): Xaa can be any naturally occurring amino acid
  misc_feature (32)..(33): Xaa can be any naturally occurring amino acid

SEQ ID NO: 62 - protein, 58 aa, ARTIFICIAL SEQUENCE
  Engineered PDL1 binding polypeptide
  misc_feature (11)..(11): Xaa can be any naturally occurring amino acid
  misc_feature (13)..(13): Xaa can be any naturally occurring amino acid
  misc_feature (17)..(18): Xaa can be any naturally occurring amino acid
  misc_feature (23)..(25): Xaa can be any naturally occurring amino acid
  misc_feature (27)..(27): Xaa can be any naturally occurring amino acid
  misc_feature (32)..(33): Xaa can be any naturally occurring amino acid
VDAKYAKERTXAXWEIXXLPNLXXXQXGAFIXXLHDDPSQSSELLSEAKKLSESQAPK

SEQ ID NO: 63 - protein, 58 aa, ARTIFICIAL SEQUENCE
  Engineered PDL1 binding polypeptide
  misc_feature (11)..(11): Xaa can be any naturally occurring amino acid
  misc_feature (13)..(13): Xaa can be any naturally occurring amino acid
  misc_feature (17)..(18): Xaa can be any naturally occurring amino acid
  misc_feature (23)..(25): Xaa can be any naturally occurring amino acid
  misc_feature (27)..(27): Xaa can be any naturally occurring amino acid
  misc_feature (32)..(33): Xaa can be any naturally occurring amino acid
VDAKYAKERTXAXWEIXXLPNLXXXQXGAFIXXLHDDPSQSSELLAEAKKLSEAQAPK

SEQ ID NO: 64 - protein, 58 aa, ARTIFICIAL SEQUENCE
  Engineered PDL1 binding polypeptide
  misc_feature (11)..(11): Xaa can be any naturally occurring amino acid
  misc_feature (13)..(13): Xaa can be any naturally occurring amino acid
  misc_feature (17)..(18): Xaa can be any naturally occurring amino acid
  misc_feature (23)..(25): Xaa can be any naturally occurring amino acid
  misc_feature (27)..(27): Xaa can be any naturally occurring amino acid
  misc_feature (32)..(33): Xaa can be any naturally occurring amino acid
VDAKYAKERTXAXWEIXXLPNLXXXQXGAFIXXLHDQPEQSSELLSEAKKLSESQAPK

SEQ ID NO: 65 - protein, 58 aa, ARTIFICIAL SEQUENCE
  Engineered PDL1 binding polypeptide
  misc_feature (11)..(11): Xaa can be any naturally occurring amino acid
  misc_feature (13)..(13): Xaa can be any naturally occurring amino acid
  misc_feature (17)..(18): Xaa can be any naturally occurring amino acid
  misc_feature (23)..(25): Xaa can be any naturally occurring amino acid
  misc_feature (27)..(27): Xaa can be any naturally occurring amino acid
  misc_feature (32)..(33): Xaa can be any naturally occurring amino acid
VDAKYAKERTXAXWEIXXLPNLXXXQXGAFIXXLHDDPSQSSELLSEAKKLESSQAPK

SEQ ID NO: 66 - protein, 58 aa, ARTIFICIAL SEQUENCE
  Engineered PDL1 binding polypeptide
  misc_feature (11)..(11): Xaa can be any naturally occurring amino acid
  misc_feature (13)..(13): Xaa can be any naturally occurring amino acid
  misc_feature (17)..(18): Xaa can be any naturally occurring amino acid
  misc_feature (23)..(25): Xaa can be any naturally occurring amino acid
  misc_feature (27)..(27): Xaa can be any naturally occurring amino acid
  misc_feature (32)..(33): Xaa can be any naturally occurring amino acid
VDAKYAKERTXAXWEIXXLPNLXXXQXGAFIXXLHDDPSQSSELLAEAKKLESAQAPK

SEQ ID NO: 67 - protein, 58 aa, ARTIFICIAL SEQUENCE
  Engineered PDL1 binding polypeptide
  misc_feature (11)..(11): Xaa can be any naturally occurring amino acid
  misc_feature (13)..(13): Xaa can be any naturally occurring amino acid
  misc_feature (17)..(18): Xaa can be any naturally occurring amino acid
  misc_feature (23)..(25): Xaa can be any naturally occurring amino acid
  misc_feature (27)..(27): Xaa can be any naturally occurring amino acid
  misc_feature (32)..(33): Xaa can be any naturally occurring amino acid
VDAKYAKERTXAXWEIXXLPNLXXXQXGAFIXXLHDQPEQSSELLSEAKKLESSQAPK

SEQ ID NO: 68 - protein, 58 aa, ARTIFICIAL SEQUENCE
  Engineered PDL1 binding polypeptide
  misc_feature (11)..(11): Xaa can be any naturally occurring amino acid
  misc_feature (13)..(13): Xaa can be any naturally occurring amino acid
  misc_feature (17)..(18): Xaa can be any naturally occurring amino acid
  misc_feature (23)..(25): Xaa can be any naturally occurring amino acid
  misc_feature (27)..(27): Xaa can be any naturally occurring amino acid
  misc_feature (32)..(33): Xaa can be any naturally occurring amino acid
VDAKYAKERTXAXWEIXXLPNLXXXQXGAFIXXLHDDPSQSSELLSEAKKLSDSQAPK

SEQ ID NO: 69 - protein, 58 aa, ARTIFICIAL SEQUENCE
  Engineered PDL1 binding polypeptide
  misc_feature (11)..(11): Xaa can be any naturally occurring amino acid
  misc_feature (13)..(13): Xaa can be any naturally occurring amino acid
  misc_feature (17)..(18): Xaa can be any naturally occurring amino acid
  misc_feature (23)..(25): Xaa can be any naturally occurring amino acid
  misc_feature (27)..(27): Xaa can be any naturally occurring amino acid
  misc_feature (32)..(33): Xaa can be any naturally occurring amino acid
VDAKYAKERTXAXWEIXXLPNLXXXQXGAFIXXLHDDPSQSSELLAEAKKLSDSQAPK

SEQ ID NO: 70 - protein, 58 aa, ARTIFICIAL SEQUENCE
  Engineered PDL1 binding polypeptide
  misc_feature (11)..(11): Xaa can be any naturally occurring amino acid
  misc_feature (13)..(13): Xaa can be any naturally occurring amino acid
  misc_feature (17)..(18): Xaa can be any naturally occurring amino acid
  misc_feature (23)..(25): Xaa can be any naturally occurring amino acid
  misc_feature (27)..(27): Xaa can be any naturally occurring amino acid
  misc_feature (32)..(33): Xaa can be any naturally occurring amino acid
VDAKYAKERTXAXWEIXXLPNLXXXQXGAFIXXLHDDPSQSSELLAEAKKLSDAQAPK

SEQ ID NO: 71 - protein, 58 aa, ARTIFICIAL SEQUENCE
  Engineered PDL1 binding polypeptide
  misc_feature (11)..(11): Xaa can be any naturally occurring amino acid
  misc_feature (13)..(13): Xaa can be any naturally occurring amino acid
  misc_feature (17)..(18): Xaa can be any naturally occurring amino acid
  misc_feature (23)..(25): Xaa can be any naturally occurring amino acid
  misc_feature (27)..(27): Xaa can be any naturally occurring amino acid
  misc_feature (32)..(33): Xaa can be any naturally occurring amino acid
VDAKYAKERTXAXWEIXXLPNLXXXQXGAFIXXLHDQPEQSSELLSEAKKLSDSQAPK

SEQ ID NO: 72 - protein, 58 aa, ARTIFICIAL SEQUENCE
  Engineered PDL1 binding polypeptide
  misc_feature (11)..(11): Xaa can be any naturally occurring amino acid
  misc_feature (13)..(13): Xaa can be any naturally occurring amino acid
  misc_feature (17)..(18): Xaa can be any naturally occurring amino acid
  misc_feature (23)..(25): Xaa can be any naturally occurring amino acid
  misc_feature (27)..(27): Xaa can be any naturally occurring amino acid
  misc_feature (32)..(33): Xaa can be any naturally occurring amino acid
VDAKYAKERTXAXWEIXXLPNLXXXQXGAFIXXLHDDPSQSSELLAEAKKLNKAQAPK

SEQ ID NO: 73 - protein, 58 aa, ARTIFICIAL SEQUENCE
  Engineered PDL1 binding polypeptide
  misc_feature (11)..(11): Xaa can be any naturally occurring amino acid
  misc_feature (13)..(13): Xaa can be any naturally occurring amino acid
  misc_feature (17)..(18): Xaa can be any naturally occurring amino acid
  misc_feature (23)..(25): Xaa can be any naturally occurring amino acid
  misc_feature (27)..(27): Xaa can be any naturally occurring amino acid
  misc_feature (32)..(33): Xaa can be any naturally occurring amino acid
AEAKYAKERTXAXWEIXXLPNLXXXQXGAFIXXLHDDPSQSSELLAEAKKLNKAQAPK

SEQ ID NO: 74 - protein, 58 aa, ARTIFICIAL SEQUENCE
  Engineered PDL1 binding polypeptide
  misc_feature (11)..(11): Xaa can be any naturally occurring amino acid
  misc_feature (13)..(13): Xaa can be any naturally occurring amino acid
  misc_feature (17)..(18): Xaa can be any naturally occurring amino acid
  misc_feature (23)..(25): Xaa can be any naturally occurring amino acid
  misc_feature (27)..(27): Xaa can be any naturally occurring amino acid
  misc_feature (32)..(33): Xaa can be any naturally occurring amino acid
ADAKYAKERTXAXWEIXXLPNLXXXQXGAFIXXLHDDPSQSSELLSEAKKLNDSQAPK